European Patent Specification EP 3 310 169 B1, published May 17, 2023. Title: METHODS FOR MODULATING RNA SPLICING. Applicant: PTC THERAPEUTICS, INC. Application PCT/US2016/34864. The sequence listing filed with the application follows.

SEQUENCE LISTING (120 sequences)

SEQ ID NO: 1 - RNA, 8 nt, Artificial Sequence
  A variant of recognition element for splicing modifier(REMS)
  misc_feature 6, 8: n = A,U,C or G
gagurngn

SEQ ID NO: 2 - RNA, 8 nt, Artificial Sequence
  A variant of recognition element for splicing modifier(REMS)
gaguragu

SEQ ID NO: 3 - RNA, 10 nt, Artificial Sequence
  A variant of recognition element for splicing modifier(REMS)
  misc_feature 2, 8, 10: n = A,T,C or G
angagurngn

SEQ ID NO: 4 - RNA, 10 nt, Artificial Sequence
  A variant of recognition element for splicing modifier(REMS)
  misc_feature 2: n = A,T,C or G
angaguragu

SEQ ID NO: 5 - DNA, 8 bp, Artificial Sequence
  nucleotide sequence of a non-endogenous REMS introduced into the nucleotide sequence of the artificial gene construct
  misc_feature 6, 8: n = A,T,C or G
gagtrngn

SEQ ID NO: 6 - DNA, 8 bp, Artificial Sequence
  A variant of recognition element for splicing modifier(REMS)
gagtragt

SEQ ID NO: 7 - DNA, 10 bp, Artificial Sequence
  A variant of recognition element for splicing modifier(REMS)
  misc_feature 2, 8, 10: n = A,T,C or G
angagtrngn

SEQ ID NO: 8 - DNA, 10 bp, Artificial Sequence
  A variant of recognition element for splicing modifier(REMS)
  misc_feature 2: n = A,T,C or G
angagtragt

SEQ ID NO: 9 - DNA, 4 bp, Artificial Sequence
  A nucleotide sequence has affinity with U1 snRNP
  misc_feature 2: n = A,T,C or G
anga

SEQ ID NO: 10 - DNA, 28 bp, Artificial Sequence
  Forward primer used for preparing SNM2 minigene construct
cgcggatccataattcccccaccacctc

SEQ ID NO: 11 - DNA, 28 bp, Artificial Sequence
  Reverse primer used for preparing SNM2 minigene construct
cgcggatccgtgctgctctatgccagca

SEQ ID NO: 12 - DNA, 21 bp, Artificial Sequence
  Forward primer used for amplifying only transcripts derived from the transfected plasmids
gatgctgatgctttgggaagt

SEQ ID NO: 13 - DNA, 19 bp, Artificial Sequence
  primer used for identifying alternatively spliced mRNAs -APLP2e6F1
acggcaccatgtcagacaa

SEQ ID NO: 14 - DNA, 20 bp, Artificial Sequence
  Primer used for identifying alternatively spliced mRNAs - APLP2e8R1
caacatcattggttggcaga

SEQ ID NO: 15 - DNA, 21 bp, Artificial Sequence
  Primer used for identifying alternatively spliced mRNAs - STRN3e7F1
actgctgaagatggtgaagga

SEQ ID NO: 16 - DNA, 23 bp, Artificial Sequence
  Primer used for identifying alternatively spliced mRNAs - STRN3e9R1
ccagatcagctatcatgtcgtag

SEQ ID NO: 17 - DNA, 19 bp, Artificial Sequence
  Primer used for identifying alternatively spliced mRNAs - RCC1e3F1
agacgatctgcacttcgca

SEQ ID NO: 18 - DNA, 21 bp, Artificial Sequence
  Primer used for identifying alternatively spliced mRNAs - RCC1e5e6R1
gtgagaccttcaccttcttgc

SEQ ID NO: 19 - DNA, 23 bp, Artificial Sequence
  Primer used for identifying alternatively spliced mRNAs - ERGIC3e6F1
tgtatggcttcttggaagtcaat

SEQ ID NO: 20 - DNA, 24 bp, Artificial Sequence
  Primer used for identifying alternatively spliced mRNAs - ERGIC3e9e10R1
gtagtgggtcatgttgatgttgtc

SEQ ID NO: 21 - DNA, 22 bp, Artificial Sequence
  Primer used for identifying alternatively spliced mRNAs - SMN Rev
cgcttcacattccagatctgtc

SEQ ID NO: 22 - DNA, 17 bp, Artificial Sequence
  Primer used for identifying alternatively spliced mRNAs - FOXM1 For
gtgttgcagccctcggt

SEQ ID NO: 23 - DNA, 21 bp, Artificial Sequence
  Primer used for identifying alternatively spliced mRNAs - FOXM1 Rev
tgaactggaagcaaaggagaa

SEQ ID NO: 24 - DNA, 18 bp, Artificial Sequence
  Primer used for identifying alternatively spliced mRNAs - VPS29e1F1
cggtggtggtgactgagc

SEQ ID NO: 25 - DNA, 21 bp, Artificial Sequence
  Primer used for identifying alternatively spliced mRNAs - VPS29e3R1
gggatgtgcagatctcctaat

SEQ ID NO: 26 - DNA, 26 bp, Artificial Sequence
  Primer used for identifying alternatively spliced mRNAs - GGCTe1F1
agatgaggagagttttctgtactttg

SEQ ID NO: 27 - DNA, 20 bp, Artificial Sequence
  Primer used for identifying alternatively spliced mRNAs - GGCTe4R1
tctcttgatactccagcggc

SEQ ID NO: 28 - DNA, 23 bp, Artificial Sequence
  Primer used for identifying alternatively spliced mRNAs - PRKDC e9F1
gatctgaagagatatgctgtgcc

SEQ ID NO: 29 - DNA, 20 bp, Artificial Sequence
  Primer used for identifying alternatively spliced mRNAs - PRKDC e12R1
acggtcgtcaccagtgtctg

SEQ ID NO: 30 - DNA, 23 bp, Artificial Sequence
  Primer used for identifying alternatively spliced mRNAs - PRKDC e50F1
gggtccctaaagatgaagtgtta

SEQ ID NO: 31 - DNA, 22 bp, Artificial Sequence
  Primer used for identifying alternatively spliced mRNAs - PRKDC e52R1
attcaccaaagcctggaagtat

SEQ ID NO: 32 - DNA, 24 bp, Artificial Sequence
  Primer used for identifying alternatively spliced mRNAs - MADD e20F1
cagaaagtgtaaataccccagttg

SEQ ID NO: 33 - DNA, 19 bp, Artificial Sequence
  Primer used for identifying alternatively spliced mRNAs - MADD e22R1
gctcacaccactgtctgcg

SEQ ID NO: 34 - DNA, 22 bp, Artificial Sequence
  Primer used for identifying alternatively spliced mRNAs - LARP7 5'UTRF1
cttccttggcttcgagtctctc

SEQ ID NO: 35 - DNA, 25 bp, Artificial Sequence
  Primer used for identifying alternatively spliced mRNAs - LARP7 e2R1
cctgtgtcctatcatttgttttctc

SEQ ID NO: 36 - DNA, 23 bp, Artificial Sequence
  Primer used for identifying alternatively spliced mRNAs - LARP7 e1F1
cgaaagtaaccgagactatcagg

SEQ ID NO: 37 - DNA, 22 bp, Artificial Sequence
  Primer used for identifying alternatively spliced mRNAs - LARP7 e4R1
ttcagtgctttcttcttccatt

SEQ ID NO: 38 - DNA, 19 bp, Artificial Sequence
  Primer used for identifying alternatively spliced mRNAs - ARMCX6 e2F1
cggcacaagtttcagcgag

SEQ ID NO: 39 - DNA, 22 bp, Artificial Sequence
  Primer used for identifying alternatively spliced mRNAs - ARMCX6 e4R1
cagggtgagtaaggatggaggg

SEQ ID NO: 40 - DNA, 21 bp, Artificial Sequence
  Primer used for identifying alternatively spliced mRNAs - GALC e4F1
ggatacgagtggtggttgatg

SEQ ID NO: 41 - DNA, 23 bp, Artificial Sequence
  Primer used for identifying alternatively spliced mRNAs - GALC e7R1
cagagatggactcccagagatta

SEQ ID NO: 42 - DNA, 20 bp, Artificial Sequence
  Primer used for identifying alternatively spliced mRNAs - LAMA2 e4F1
ggattttggaacgctctctt

SEQ ID NO: 43 - DNA, 26 bp, Artificial Sequence
  Primer used for identifying alternatively spliced mRNAs - LAMA2 e6R1
gaaatatccttgaccgagtagtaata

SEQ ID NO: 44 - DNA, 22 bp, Artificial Sequence
  Primer used for identifying alternatively spliced mRNAs - ABHD10e4F1
gagaaggtcgtggctcttattg

SEQ ID NO: 45 - DNA, 23 bp, Artificial Sequence
  Primer used for identifying alternatively spliced mRNAs - ABHD10e6R1
gggctatgtaacaagcagtgatg

SEQ ID NO: 46 - DNA, 19 bp, Artificial Sequence
  Primer used for identifying alternatively spliced mRNAs - FADS2e5F1
ctgccaactggtggaatca

SEQ ID NO: 47 - DNA, 22 bp, Artificial Sequence
  Primer used for identifying alternatively spliced mRNAs - FADS2e8R1
gatgccgtagaaagggatgtag

SEQ ID NO: 48 - DNA, 21 bp, Artificial Sequence
  Primer used for identifying alternatively spliced mRNAs - DIAPH3e10F1
tcaatgccctggttacatctc

SEQ ID NO: 49 - DNA, 24 bp, Artificial Sequence
  Primer used for identifying alternatively spliced mRNAs - DIAPH3e13R1
acaatctgggatacacactcatca

SEQ ID NO: 50 - DNA, 24 bp, Artificial Sequence
  Primer used for identifying alternatively spliced mRNAs - PDIA3e3F1
ctgccaacactaacacctgtaata

SEQ ID NO: 51 - DNA, 22 bp, Artificial Sequence
  Primer used for identifying alternatively spliced mRNAs - PDIA3e7R1
agtccttgccctgtatcaaatc

SEQ ID NO: 52 - DNA, 21 bp, Artificial Sequence
  Primer used for identifying alternatively spliced mRNAs - FN1e34F1
gctcatccgtggttgtatcag

SEQ ID NO: 53 - DNA, 23 bp, Artificial Sequence
  Primer used for identifying alternatively spliced mRNAs - FN1e36R1
gatcgtctcagtcttggttctcc

SEQ ID NO: 54 - DNA, 21 bp, Artificial Sequence
  Primer used for identifying alternatively spliced mRNAs - PARP1e20F1
agtgccaactactgccatacg

SEQ ID NO: 55 - DNA, 23 bp, Artificial Sequence
  Primer used for identifying alternatively spliced mRNAs - PARP1ee23R1
aatcctttctgaggtggtttagt

SEQ ID NO: 56 - DNA, 20 bp, Artificial Sequence
  Primer used for identifying alternatively spliced mRNAs - COL1Ae2F1
caaggtgttgtgcgatgacg

SEQ ID NO: 57 - DNA, 26 bp, Artificial Sequence
  Primer used for identifying alternatively spliced mRNAs - COL1Ae6R1
ggttgatttctcatcatagccataag

SEQ ID NO: 58 - DNA, 20 bp, Artificial Sequence
  Primer used for identifying alternatively spliced mRNAs - COLA1e7F1
cctctggtcctcgtggtctc

SEQ ID NO: 59 - DNA, 20 bp, Artificial Sequence
  Primer used for identifying alternatively spliced mRNAs - COL1Ae12R1
ccatccaaaccactgaaacc

SEQ ID NO: 60 - DNA, 19 bp, Artificial Sequence
  Primer used for identifying alternatively spliced mRNAs - COLA1e27F1
ggtcctgctggcaaagatg

SEQ ID NO: 61 - DNA, 18 bp, Artificial Sequence
  Primer used for identifying alternatively spliced mRNAs - COLA1e31R1
gctcgccagggaaacctc

SEQ ID NO: 62 - DNA, 19 bp, Artificial Sequence
  Primer used for identifying alternatively spliced mRNAs - COLA1e31F1
aggcgagagaggtttccct

SEQ ID NO: 63 - DNA, 21 bp, Artificial Sequence
  Primer used for identifying alternatively spliced mRNAs - COLA1e33e34R1
ggaccactttcacccttgtca

SEQ ID NO: 64 - DNA, 19 bp, Artificial Sequence
  Primer used for identifying alternatively spliced mRNAs - COLA1e47F1
gggcgacagaggcataaag

SEQ ID NO: 65 - DNA, 20 bp, Artificial Sequence
  Primer used for identifying alternatively spliced mRNAs - COLA1e48R1
tcacggtcacgaaccacatt

SEQ ID NO: 66 - DNA, 22 bp, Artificial Sequence
  Primer used for identifying alternatively spliced mRNAs - COL1A2e20F1
caaaggagagagcggtaacaag

SEQ ID NO: 67 - DNA, 22 bp, Artificial Sequence
  Primer used for identifying alternatively spliced mRNAs - COL1A2e22R1
aagaccacgagaaccaggacta

SEQ ID NO: 68 - DNA, 19 bp, Artificial Sequence
  Primer used for identifying alternatively spliced mRNAs - COL1A2e22F1
cctggttctcgtggtcttc

SEQ ID NO: 69 - DNA, 18 bp, Artificial Sequence
  Primer used for identifying alternatively spliced mRNAs - COL1A2e24e25R1
gccgacaggaccttcttt

SEQ ID NO: 70 - DNA, 19 bp, Artificial Sequence
  Primer used for identifying alternatively spliced mRNAs - COL1A2e29F1
tggcaaaccaggagaaagg

SEQ ID NO: 71 - DNA, 20 bp, Artificial Sequence
  Primer used for identifying alternatively spliced mRNAs - COL1A2e31R1
aaggacctcggcttccaata

SEQ ID NO: 72 - DNA, 18 bp, Artificial Sequence
  Primer used for identifying alternatively spliced mRNAs - COL3A1e7e8F1
ggcaagctggtccttcag

SEQ ID NO: 73 - DNA, 19 bp, Artificial Sequence
  Primer used for identifying alternatively spliced mRNAs - COL3A1e11R1
ggagcacctgtttcaccct

SEQ ID NO: 74 - DNA, 23 bp, Artificial Sequence
  Primer used for identifying alternatively spliced mRNAs - COL3A1e45F1
tgacaaaggtgaaacaggtgaac

SEQ ID NO: 75 - DNA, 20 bp, Artificial Sequence
  Primer used for identifying alternatively spliced mRNAs - COL3A1e47R1
gtccactgggtccaacaggt

SEQ ID NO: 76 - DNA, 20 bp, Artificial Sequence
  Primer used for identifying alternatively spliced mRNAs - COL5A2e10e11F1
aatgggtccgattggttcac

SEQ ID NO: 77 - DNA, 22 bp, Artificial Sequence
  Primer used for identifying alternatively spliced mRNAs - COL52Ae16R1
caagtctccctctctctcctgg

SEQ ID NO: 78 - DNA, 21 bp, Artificial Sequence
  Primer used for identifying alternatively spliced mRNAs - COL52Ae30F1
ggtgaaagaggagaacaagga

SEQ ID NO: 79 - DNA, 20 bp, Artificial Sequence
  Primer used for identifying alternatively spliced mRNAs - COL52Ae33R1
tcaccagggagtccagttat

SEQ ID NO: 80 - DNA, 22 bp, Artificial Sequence
  Primer used for identifying alternatively spliced mRNAs - COL52Ae33F1
agaacctgggataactggactc

SEQ ID NO: 81 - DNA, 21 bp, Artificial Sequence
  Primer used for identifying alternatively spliced mRNAs - COL5A2e35e36R1
agacctcttgcaccatcattt

SEQ ID NO: 82 - DNA, 17 bp, Artificial Sequence
  Primer used for identifying alternatively spliced mRNAs - COL5A2e33F1
agggaatggctggagga

SEQ ID NO: 83 - DNA, 19 bp, Artificial Sequence
  Primer used for identifying alternatively spliced mRNAs - COL5A2e36R1
cccaaaggacctggaagac

SEQ ID NO: 84 - DNA, 20 bp, Artificial Sequence
  Primer used for identifying alternatively spliced mRNAs - COL5A2e48F1
aggacctcgtggtgacaaag

SEQ ID NO: 85 - DNA, 20 bp, Artificial Sequence
  Primer used for identifying alternatively spliced mRNAs - COL5A2e50R1
gcccagggtttccttcttta

SEQ ID NO: 86 - DNA, 23 bp, Artificial Sequence
  Primer used for identifying alternatively spliced mRNAs - SMNe4F1
gatgaaagtgagaactccaggtc

SEQ ID NO: 87 - DNA, 21 bp, Artificial Sequence
  Primer used for identifying alternatively spliced mRNAs - SMNe6R1
caaagcatcagcatcatcaag

SEQ ID NO: 88 - RNA, 10 nt, Artificial Sequence
  sequence motif resulted in a compound-dependent increase in the inclusion of exon 7 of SMN2
aggaguaagu

SEQ ID NO: 89 - DNA, 10 bp, Artificial Sequence
  sequence motif resulted in selectivity against the inclusion of exon 7A of FOXM1
atcagtaagt

SEQ ID NO: 90 - DNA, 10 bp, Artificial Sequence
  Alternative splicing sequence motif which affected exon 7A Delta-C of gene FOXM1, or exon 7 of APLP2
atgagtaagt

SEQ ID NO: 91 - DNA, 4 bp, Artificial Sequence
  sequence motif resulted in a compound-dependent increase in the inclusion of exon 7 of APLP2, exon 2 of GGCT, or exon 5 of ABHD10
atga

SEQ ID NO: 92 - DNA, 4 bp, Artificial Sequence
  sequence motif resulted in a compound-dependent increase in the inclusion of exon 8 of STRN3, exon 2 of LARP7, or exon 30 of COL1A1
aaga

SEQ ID NO: 93 - DNA, 4 bp, Artificial Sequence
  sequence motif resulted in a compound-dependent increase in the inclusion of exon 2 of VPS29 or exon 21 of MADD
caga

SEQ ID NO: 94 - DNA, 4 bp, Artificial Sequence
  sequence motif resulted in a compound-dependent increase in the inclusion of exon 8 of ERGIC3
gaga

SEQ ID NO: 95 - DNA, 4 bp, Artificial Sequence
  sequence motif resulted in a compound-dependent increase in the inclusion of part of exon 1 of LARP7
cgga

SEQ ID NO: 96 - DNA, 10 bp, Artificial Sequence
  Alternative splicing sequence motif which affected exon 7 of gene SMN2, or exon 5 of COL1A1
aggagtaagt

SEQ ID NO: 97 - DNA, 10 bp, Artificial Sequence
  Alternative splicing sequence motif which affected exon 2 of gene GGCT
atgagtaggt

SEQ ID NO: 98 - DNA, 10 bp, Artificial Sequence
  Alternative splicing sequence motif which affected exon 5 of gene ABHD10
atgagtatgt

SEQ ID NO: 99 - DNA, 10 bp, Artificial Sequence
  Alternative splicing sequence motif which affected exon 8 of gene STRN3, exon 30 of COL1A1, exon 5 of LAMA2, exon 30 of COL1A2, exon 35 of COL5A2, or exon 49 of COL5A2
aagagtaagt

SEQ ID NO: 100 - DNA, 10 bp, Artificial Sequence
  Alternative splicing sequence motif which affected exon 2 of gene VPS29, exon 32 of COL1A1, exon 22 of COL1A2, exon 10 of COL3A1, exon 46 of COL3A1, or exon 34 of COL5A2
cagagtaagt

SEQ ID NO: 101 - DNA, 10 bp, Artificial Sequence
  Alternative splicing sequence motif which affected exon 8 of gene ERGIC3, or exon 35 of FN1
gagagtaagt

SEQ ID NO: 102 - DNA, 10 bp, Artificial Sequence
  Alternative splicing sequence motif which affected exon 21 of gene MADD
cagagtaagg

SEQ ID NO: 103 - DNA, 10 bp, Artificial Sequence
  Alternative splicing sequence motif which affected exon 1 of gene LARP7
cggagtaagt

SEQ ID NO: 104 - DNA, 10 bp, Artificial Sequence
  Alternative splicing sequence motif which affected exon 2 of gene LARP7
aagagtaaga

SEQ ID NO: 105 - DNA, 10 bp, Artificial Sequence
  Alternative splicing sequence motif which affected exon 3 of gene ARMCX6
tagagtatga

SEQ ID NO: 106 - DNA, 10 bp, Artificial Sequence
  Alternative splicing sequence motif which affected exon 5 of gene GALC
tggagttagt

SEQ ID NO: 107 - DNA, 10 bp, Artificial Sequence
  Alternative splicing sequence motif which affected exon 11 of gene PRKDC
aggagtatgt

SEQ ID NO: 108 - DNA, 10 bp, Artificial Sequence
  Alternative splicing sequence motif which affected exon 51 of gene PRKDC
gcgagtacgt

SEQ ID NO: 109 - DNA, 10 bp, Artificial Sequence
  Alternative splicing sequence motif which affected exon 4 of gene RCC1
agaggtaaga

SEQ ID NO: 110 - DNA, 10 bp, Artificial Sequence
  Alternative splicing sequence motif which affected exon 6 of gene FADS2
ctgagtaagt

SEQ ID NO: 111 - DNA, 10 bp, Artificial Sequence
  Alternative splicing sequence motif which affected exon 11 of gene DIAPH3
ttgaatatcc

SEQ ID NO: 112 - DNA, 10 bp, Artificial Sequence
  Alternative splicing sequence motif which affected exon 35 of gene PARP1
acgagtatcc

SEQ ID NO: 113 - DNA, 10 bp, Artificial Sequence
  Alternative splicing sequence motif which affected exon 11 of gene COL1A1
cagagtgagt

SEQ ID NO: 114 - DNA, 10 bp, Artificial Sequence
  Alternative splicing sequence motif which affected exon 46 of gene COL1A1 or exon 13 of COL5A2
ccgagtaagt

SEQ ID NO: 115 - DNA, 10 bp, Artificial Sequence
  Alternative splicing sequence motif which affected exon 21 of gene COL1A2
gagagtaggt

SEQ ID NO: 116 - DNA, 10 bp, Artificial Sequence
  Alternative splicing sequence motif which affected exon 32 of gene COL5A2
tagagtaagt

SEQ ID NO: 117 - DNA, 10 bp, Artificial Sequence
  Alternative splicing sequence motif which affected exon 5 of gene SMN2
accagtaagt

SEQ ID NO: 118 - RNA, 23 nt, Artificial Sequence
  TSL2 (terminal stem loop 2) in SMN2
auuccuuaaauuaaggaguaagu

SEQ ID NO: 119 - RNA, 23 nt, Artificial Sequence
  Sequence illustrating examplary mutations introduced into TSL2 in SMN2
auuccauaaauuauggaguaagu

SEQ ID NO: 120 - RNA, 9 nt, Artificial Sequence
  Sequence illustrating examplary mutations introduced into TSL2 in SMN2
acuuaccug